European Patent Application EP 4 803 623 A1, published September 9, 2026. Title: USE OF HIGH-ACTIVITY AND THERMOSTABLE RIBONUCLEASE SIRE_0902 IN SPECIFIC RECOGNITION OF GG SITES. Applicant: BestEnzymes Biotech Co., Ltd. Application EP. The sequence listing filed with the application follows.

SEQUENCE LISTING (9 sequences)

SEQ ID NO: 1 - DNA, 387 bp, synthetic construct
  source 1..387: mol_type = other DNA
atgaactataaagaatggatagagcaagctttggaagatctcgacactgcaaaacttcttttaactaatgggaaatattacgcttctgccttctattctcagcaagcagtagagaaatcattaaagtcccttataatttatcttggaaaagatcctggtaagacgcattcacttactgaacttattgaaatggtagagaaggaaggagtgactatgccaataaatattaaagagaatctgatggttctttcaccccatttcataatttcaagatatccagacgctgcaaacggagttccctttaagcagtatagtaaatcaatttctgaggacctttataatagagcaaaagaggtgattgaatgggtaaaggaaaatctgcaatag

SEQ ID NO: 2 - protein, 128 aa, synthetic construct
MNYKEWIEQALEDLDTAKLLLTNGKYYASAFYSQQAVEKSLKSLIIYLGKDPGKTHSLTELIEMVEKEGVTMPINIKENLMVLSPHFIISRYPDAANGVPFKQYSKSISEDLYNRAKEVIEWVKENLQ

SEQ ID NO: 3 - DNA, 345 bp, synthetic construct
  source 1..345: mol_type = other DNA
atgggtaaaggaaaatctgcaatagagagccaaatgaagttaataaatctagtaaaggaaatagtggaagaaatagctaaggacttccagcagttagacgaagtttatatctttggctctagagctaaaggaaattatttagatactagtgatatagatgttatcttcgttttcaagggcataaaggaaatgaacgtatttgataggatgtatatggtaagtaaatacataaaaggaaatatagattatatagtattaaacgaggacgaaaaggatagaataagagagaagaaattattttggaagaggaataagggatttgtagatataaaggaatttctataa

SEQ ID NO: 4 - protein, 114 aa, synthetic construct
MGKGKSAIESQMKLINLVKEIVEEIAKDFQQLDEVYIFGSRAKGNYLDTSDIDVIFVFKGIKEMNVFDRMYMVSKYIKGNIDYIVLNEDEKDRIREKKLFWKRNKGFVDIKEFL

SEQ ID NO: 5 - DNA, 52 bp, synthetic construct
  source 1..52: mol_type = other DNA
ggaattccatatgcaccaccaccaccaccacaactataaagaatggatagag

SEQ ID NO: 6 - DNA, 32 bp, synthetic construct
  source 1..32: mol_type = other DNA
acgcgtcgacttatagaaattcctttatatct

SEQ ID NO: 7 - RNA, 46 nt, synthetic construct
  source 1..46: mol_type = other RNA
tgttaagtctggtttccctccagggatctaagcttgaacccccccc

SEQ ID NO: 8 - DNA, 59 bp, synthetic construct
  source 1..59: mol_type = other DNA
ttcgagctcggtacccggttgatagggaacaagacgaatagggatcctctagagtcgac

SEQ ID NO: 9 - DNA, 117 bp, synthetic construct
  source 1..117: mol_type = other DNA
ttcgagctcggtacccggttgatagggaacaagacgaatagggatcctctagagtcgacaagctcgagccatgggccaactatcctgttctgcttatccctaggagatctcgagctg